European Patent Application EP 4 487 918 A2, published January 8, 2025. Title: Amphiphilic polymers and their use for improved production of nanoparticles for the targeted delivery of antigens. Applicant: Topas Therapeutics GmbH. The sequence listing filed with the application follows.

SEQUENCE LISTING (3 sequences)

SEQ ID NO: 1 - protein, 15 aa, Homo sapiens
  REGION 1..15: note = peptide comprising T cell epitope
LNSKIAFKIVSQEPA

SEQ ID NO: 2 - protein, 15 aa, Homo sapiens
  REGION 1..15: note = peptide comprising T cell epitope
TPMFLLSRNTGEVRT

SEQ ID NO: 3 - protein, 15 aa, Homo sapiens
  REGION 1..15: note = peptide comprising T cell epitope
REGIAFRPASKTFTV